European Patent Application EP 4 286 535 A1, published December 6, 2023. Title: METHOD AND DETECTION KIT FOR THE DETECTION OF PYROGENS IN BIOLOGICAL SAM-PLES. Applicant: Minerva Biolabs GmbH. Application unknown. The sequence listing filed with the application follows.

SEQUENCE LISTING (18 sequences)

SEQ ID NO: 1 - DNA, 20 bp, Artificial Oligonukleotid
  Primer
cacgctatcgctgcctctat

SEQ ID NO: 2 - DNA, 22 bp, Artificial Oligonukleotid
  Primer
cggctattgagatacactgatc

SEQ ID NO: 3 - DNA, 18 bp, Artificial Oligonukleotid
  probe
agctatcacgctcatgcg

SEQ ID NO: 4 - DNA, 21 bp, Artificial Oligonukleotid
  Primer
atctttgaagaagaacctatc

SEQ ID NO: 5 - DNA, 16 bp, Artificial Oligonukleotid
  Primer
ctgtgagtcccggagc

SEQ ID NO: 6 - DNA, 23 bp, Artificial Oligonukleotid
  probe
taacgaggcttatgtgcacgatg

SEQ ID NO: 7 - DNA, 21 bp, Artificial Oligonukleotid
  Primer
ctttcagagacagcagagcac

SEQ ID NO: 8 - DNA, 22 bp, Artificial Oligonukleotid
  Primer
cttggcaaaactgcaccttcac

SEQ ID NO: 9 - DNA, 18 bp, Artificial Oligonukleotid
  probe
cgtggctctcttggcagc

SEQ ID NO: 10 - DNA, 23 bp, Artificial Oligonukleotid
  Primer
catgtaacaagagtaacatgtgt

SEQ ID NO: 11 - DNA, 20 bp, Artificial Oligonukleotid
  Primer
caccaggcaagtctcctcat

SEQ ID NO: 12 - DNA, 22 bp, Artificial Oligonukleotid
  probe
agccatctttggaaggttcagg

SEQ ID NO: 13 - DNA, 20 bp, Artificial Oligonukleotid
  Primer
ctttgcagtgacccagcatc

SEQ ID NO: 14 - DNA, 21 bp, Artificial Oligonukleotid
  Primer
tcttggcaaaccagaaaccct

SEQ ID NO: 15 - DNA, 27 bp, Artificial Oligonukleotid
  probe
ctgtttcttggcgtgtgaagataaccc

SEQ ID NO: 16 - DNA, 19 bp, Artificial Oligonukleotid
  Primer
tgcttgttcctcagcctct

SEQ ID NO: 17 - DNA, 20 bp, Artificial Oligonukleotid
  Primer
cttgagggtttgctacaaca

SEQ ID NO: 18 - DNA, 20 bp, Artificial Oligonukleotid
  probe
acgctcttctgcctgctgca